European Patent Specification EP 3 599 853 B1, published July 30, 2025. Title: HERBICIDAL COMPOSITIONS AND METHODS OF USE THEREOF. Applicant: The Regents of the University of California Yan Yan Tang Yi Jacobsen Steve E. Liu Qikun. Application Concurrently Herewith. The sequence listing filed with the application follows.

SEQUENCE LISTING (52 sequences)

SEQ ID NO: 1 - protein, 610 aa, Aspergillus terreus
MLLSQTRGRLPSLRTLKRSMAVRPLSTTLPKHKADEKEPVLNKVSRHVTQPISQGASQAMLYATGLTEADMNKAQVGISSVWYNGNPCNMHLLDLNNRVREGVQKAGLVGFQFNTVGVSDAISMGTSGMRFSLQSRDLIADSIETVMGGQWYDANISIPGCDKNMPGVLMAMGRVNRPSLMVYGGSIKPGCASMQNNADIDIVSAFQAYGQFISGEITEPQRFDIIRNACPGGGACGGMYTANTMATAIEVMGMTLPGSSSNPAESAAKNIECLAAGEAIKKLLVEDIRPSDILTRQAFENAMIVVNITGGSTNAVLHLIAIADSVGIKLDIEDFQKVSDRVPFLADLKPSGKYVMADLHKIGGTPSLLKFLLKEGLIDGSGMTVTGQTLAKNLENVPDFPEDQKIIRPLSNPIKETGHIQILRGSLAPGGSVGKITGKEGTVFTGKARVFDHEDDFIAALERKEIKKEEKTVVVIRYTGPKGGPGMPEMLKPSSALMGAGLGGSCALITDGRFSGGSHGFLIGHIVPEAAVGGPIGLVKDGDVITIDAVKRVLDLDVDETTLAERRKQWEADKEAGRLPPTGLTLRGTLGKYARNVKDASHGCITDALD

SEQ ID NO: 2 - protein, 541 aa, Aspergillus fischeri
MLYATGLEEADMNKAQVGISSVWFEGNPCNMHLMDLSLVVRDSVARAGLVPMRFNSIGVSDGISMGTSGMRYSLQSREIIADGIETVMNGQWYDANISLPGCDKNMPGVVMAMGRVNRPSIVIYGGSIKPGCSAGGQTLDLVSAFQSYGQYITGQIDEAQRFDIIRHACPGSGACGGMYTANTMATAIEVLGLTVPGSSSCPAEDPRKKAECEEIGETVKNLLKEDIRPSDILTRQAFENAMIVVNILGGSTNAVMHLIAIAQSVGIKLTIDDFQAVSDKTPFLADLKPSGKYVMHDLYKIGGTPALLRFLLKEGLIDGSGITVTGKTMKENVASWPDFPEDQPIIRPLSDPIKPTGHLQILRGSLAPGGSVGKITGKEGLRFEGSAKCYDYEDAFVDALEKGEIKKGEKTVVIIRYEGPKGGPGMPEMLKPSAAIMGAGLGQDVALLTDGRFSGGSHGFLIGHIVPEAMDGGPIALVKDGDRVIIDAEKRVVDLDISGEEMQRRKKAWKAPEPRAKKGTLKKYAALVSDASHGCVTDGPL

SEQ ID NO: 3 - protein, 609 aa, Penicillium brasilianum
MLPQTRARVPAALRSLTRSSATVRTLSTTLARFQNEDKALNKTSRTITQPKSQGASQAMLYAVGLKEEDMNKAQVGISSVWFNGNPCNMHLLDLNNKVRQGVQDQGLIGFQFNTVGVSDGMSMGTPGMRYSLQSRDLIADSVETVMGGQWYDANISIPGCDKNMPGVLMAMGRVNRPSLMVYGGTIKPGCAVTQNNADIDIVSAFQAYGQFIAKEITEPQRFDVIRHACPGEGACGGMYTANTMATAIETMGMTLPGSSSNPANSQAKYLECLAAGGAIKKLLAEDIRPRDILTRQAFENAMVVVNITGGSTNAVLHLIAIADSVGIKLTIDDFQAVSDRIPFLADLKPSGKYVMADMFAIGGTPALLKMLLKEGLIDGSGMTVTGETLAKNLEKAPDFPEDQKIIRPFSNPIKSTGHIQILRGSLAPGGSVGKITGKEGTVFTGKARVFDAEDDFVAALERNEIKKDEKTVVVIRYCGPKGGPGMPEMLKPSSALMGYGLGSSCALITDGRFSGGSHGFLIGHIVPEAATGGPIGLVNDGDVITIDADNRVLDLDVPESELAERRKDWEARKAAGKLPETGLTMRGTLGKYARNVKDASQGCITDALE

SEQ ID NO: 4 - protein, 608 aa, Arabidopsis thaliana
MQATIFSPRATLFPCKPLLPSHNVNSRRPSIISCSAQSVTADPSPPITDTNKLNKYSSRITEPKSQGGSQAILHGVGLSDDDLLKPQIGISSVWYEGNTCNMHLLKLSEAVKEGVENAGMVGFRFNTIGVSDAISMGTRGMCFSLQSRDLIADSIETVMSAQWYDGNISIPGCDKNMPGTIMAMGRLNRPGIMVYGGTIKPGHFQDKTYDIVSAFQSYGEFVSGSISDEQRKTVLHHSCPGAGACGGMYTANTMASAIEAMGMSLPYSSSIPAEDPLKLDECRLAGKYLLELLKMDLKPRDIITPKSLRNAMVSVMALGGSTNAVLHLIAIARSVGLELTLDDFQKVSDAVPFLADLKPSGKYVMEDIHKIGGTPAVLRYLLELGLMDGDCMTVTGQTLAQNLENVPSLTEGQEIIRPLSNPIKETGHIQILRGDLAPDGSVAKITGKEGLYFSGPALVFEGEESMLAAISADPMSFKGTVVVIRGEGPKGGPGMPEMLTPTSAIMGAGLGKECALLTDGRFSGGSHGFVVGHICPEAQEGGPIGLIKNGDIITIDIGKKRIDTQVSPEEMNDRRKKWTAPAYKVNRGVLYKYIKNVQSASDGCVTDE

SEQ ID NO: 5 - protein, 601 aa, Glycine max
MQSTLFNPTHSLIPTSPHSIRSNSGHASLSVRASIAVETPTETVKLNKYSSRITEPKSQGASQAVLYGVGLSEDDMAKPQVGVSSVWYEGNTCNMHLLHLSEAVRDGVAAAGMVPFRFNTVGVSDAISMGTRGMCYSLQSRDLIADSIETVMAAQWYDGNISIPGCDKNMPGTIIAMGRLNRPSIMVYGGTIKPGHFEGNTFDIVSAFQCYGEYVSGSINDDQRQNVIRNSCPGAGACGGMYTANTMASAIEAMGMSLPYSSSTPAEDPLKLDECRLAGKYLLELLKMDLKPRDIITRKSLRNAMVIVMALGGSTNAVLHLIAIAKSVGIDLTLDDFQKVSDEVPFIADLKPSGKYVMEDVHKIGGTPAVIRYLLEQGFLDGDCMTVTGKTLAENAELVPPLSNGQEIIRPVENPIKKTAHIQILYGNLAPQGSVAKITGKEGLYFSGPALVFEGEEAMIAAISEDPSSFKGKVVVIRGEGPKGGPGMPEMLTPTSAIMGAGLGKEVALLTDGRFSGGSHGFVVGHICPEAQEGGPIGLIQNGDVINVDIKNRRIDVLVSDEEMEARRKKWTAPPYKANRGALYKYIKNVTPASSGCVTDE

SEQ ID NO: 6 - protein, 591 aa, Zea mays
MQSMAPTSPSLPVAGPVPRRRLQRVRAAAVSDEPKLNKYSARITEPKSQGASQAVLYGVGLTDADLRKPQVGVSSVWYEGNTCNMHLLRLAEAVRDGVREAGMVGFRFNTVGVSDAISMGTRGMCYSLQSRDLIADSIETVMGAQHYDANISIPGCDKNMPGTIMAMGRLNRPSIMIYGGTIKPGHFQGNSYDIVSAFQCYGEYVSGSITDEQRKNVLRNSCPGAGACGGMYTANTMASAIETLGMSLPYSSSTPAEDPLKLEECRLAGKYLLELLKMDLKPKDIITEKSLRNAMVIVMALGGSTNAVLHLIAIARSVGLHLTLDDFQKVSDQVPFLADLKPSGKYVMEDLHKIGGTPAVIHYLLEQGLLDGDCMTVTAKTLAENAKIFPPLSEGQQIIRPLDNPIKPTGHIQILYGNLAPEGSVAKITGKEGLYFSGPALVFEGEESMITAISENPANFKGKVVVIRGEGPKGGPGMPEMLTPTSAIMGAGLGKECALLTDGRFSGGSHGFVVGHICPEAQEGGPIGLVQSGDIITIDVSKRVIDVDLTEQQLEERRRKWTPPPYKSTSGALWKYIKLVAPASRGCVTDE

SEQ ID NO: 7 - protein, 615 aa, Solanum lycopersicum
MQAHLLSPTIYPATTTTSPLFPKCRTHLRKPPTLTIRASSTETSTPPPQTSTSTDPSQQLNKYSSRITQPKSQGGSQAILYGVGLTDEDMNKPQIGISSVWYEGNTCNMHLLKLAEAVKEGVTEAGMVGFRFNTIGVSDAISMGTRGMCFSLQSRDLIADSIETVMSAQWYDGNIAIPGCDKNMPGTIMAMGRLNRPSIMIYGGTIKPGHFQGHTFDIVSAFQVYGEYVSGAVSDEQRMNVVRNSCPGAGACGGMYTANTMASAIEAMGMSLPYSSSTPAEDSLKLDECRLAGKYLMELLKMDLKPRDIITKKSLRNAMVVVMALGGSTNAVLHLIAIARSVGLELTLDDFQKVSDEVPFLADLKPSGKYVMEDVHKIGGTPAVIRHLLELGYMDGDCMTVTGKTLAENAKLFPSLAEGQQIIRPLSNPIKETGHIQILYGNLAPEGSVAKITGKEGLYFSGPALVFEGEEAMLAAISEDPLSFKGKVVVIRGEGPKGGPGMAEMLTPTSAIMGAGLGKDVALLTDGRFSGGSHGYVVGHICPEAQEGGPIGLVQNGDIITIDIQKKKMDVQLSDEVLEQRRKNWTPPAYKADRGVLYKYIKNVQSASKGCVTDE

SEQ ID NO: 8 - protein, 594 aa, Oryza sativa
  Japonica Group
MQSLALTSPSLPAPATASGRRRRRLERIRATAVSDEPKLNKYSARITEPKSQGASQAVLYGVGLTDADLRKPQVGVSSVWYEGNTCNMHLLRLAEAVRDGVREAGMVAFRFNTVGVSDAISMGTRGMCYSLQSRDLIADSIETVMGAQHYDANISIPGCDKNMPGTIMAMGRLNRPSIMIYGGTIKPGHFQGNSYDIVSAFQCYGEFVTGSISDEQRKNVLRNSCPGAGACGGMYTANTMASAIETMGMSLPYSSSTPAEDPLKLEECRLAGKYLLELLKMDLKPKDIITEKSLRNAMVIVMALGGSTNAVLHLIAIARSVGLQLTLDDFQKVSDQVPFLADLKPSGKYVMEDLHKIGGTPAVIHYLLEQGLLDGDCMTVTGKTLAENAKIFPPLSEGQQIIRPLDNPIKSTGHIQILYGNLAPEGSVAKITGKEGMFFSGPALVFEGEESMITAISENPANFKGKVVVIRGEGPKGGPGMPEMLTPTSAIMGAGLGKECALLTDGRFSGGSHGFVVGHICPEAQEGGPIGLVQNGDKITIDVVKRVIDVELTEAELEERRRKWTPPPHKAARGALWKYTKLVSPASRGCVTDE

SEQ ID NO: 9 - protein, 591 aa, Sorghum bicolor
MQSMALTSPSLPAAGPVTGRRLQRVRATAVSDEPKLNKYSARITEPKSQGASQAVLYGVGLTDADLRKPQVGVSSVWYEGNTCNMHLLRLAEAVRDGVREAGMVGFRFNTVGVSDAISMGTRGMCYSLQSRDLIADSIETVMGAQHYDANISIPGCDKNMPGTIMAMGRLNRPSIMIYGGTIKPGHFQGNSYDIVSAFQCYGEYVSGSITDEQRKNVLRNSCPGAGACGGMYTANTMASAIETLGMSLPYSSSTPAEDPLKLEECHLAGKYLLELLKMDLKPKDIITEKSLRNAMVIVMALGGSTNAVLHLIAIARSVGLHLTLDDFQKVSDQVPFLADLKPSGKYVMEDLHKIGGTPAVIHYLLEQGLLDGDCMTVTGKTLAENAKIFPPLSEGQQIIRPLDNPIKSTGHIQILYGNLAPEGSVAKITGKEGLFFSGPALVFEGEESMITAISENPANFKGKVVVIRGEGPKGGPGMPEMLTPTSAIMGAGLGKECALLTDGRFSGGSHGFVVGHICPEAQEGGPIGLVQSGDVITIDVSKRVIDVDLTEQQLEERRRKWTPPPYKSTRGALWKYIKLVAPASRGCVTDE

SEQ ID NO: 10 - protein, 598 aa, Aspergillus terreus
MFASRIRSRALGLHPRARFENTRLPASTTGRRYKSDETLNRVSSKITQPKSQGASQAMLYATGLTEEDMSKPQVGISSVWFEGNPCNMHLHDLSAIVRDSVHRAGLVPMRFNSVGVSDGISMGTKGMRYSLQSRELIADGIETVMNAQWYDANVSLPGCDKNMPGVLMAMGRTNRPSIMVYGGSIKPGCSAKGQKLDLVSAFQSYGQFITGQIDEKERFDIIRNACPGRGACGGMYTANTLATAIETMGMTVPGSSSCPADDPKKLVECENIGEVVKTMLREDIKPRDVLTRQAFENAMIVVNILGGSTNAVLHLIAIADSVGIKLTIDDFQAVSDKTPFLADLKPSGKYLMNDLYNIGGTPALLKYLLKEGLIDGSGITVTGKTMKENVASWPDFPADQDIIRPLSNPIKPSGHLQILRGSLAPGGSVGKITGKEGLRFEGTAKCYDYEDAFIESLERGEIKKGEKTVVIIRYEGPKGGPGMPEMLKPSAAIMGAGLGQDVALLTDGRFSGGSHGFLIGHIVPEAMEGGPIALARDGDRIVIDAEERVVDLDIPTEELEKRRKEWKAPPLRYQKGTLKKYCTLVSDASHGCVTDGPI

SEQ ID NO: 11 - protein, 624 aa, Aspergillus fischeri
MFASSIRSRALGLSPRARFENTYERTFPRIASLSLLKNRQILITIVTSRLPSSTTERRYKSDETLNRISSKITQPKSQGASQAMLYATGLTEEDMSKPQVGISSVWFEGNPCNMHLHDLSAIVRDSVLRAGLVPMRFNSVGVSDGISMGTKGMRYSLQSRELIADGIETVMNAQWYDANVSLPGCDKNMPGVLMAMGRTNRPSIMVYGGSIKPGCSAKGQKLDLVSAFQSYGQFITGQIDEKERFDIIRNACPGRGACGGMYTANTLATAIETMGMTVPGSSSCPADDPKKLVECENIGEVVKTMLREDIKPRDVLTRQAFENAMIVVNVLGGSTNAVLHLIAIADSVGIKLTIDDFQTVSDKTPFLADLKPSGKYLMNDLYNIGGTPALLKYLLKEGLIDGSGITVTGKTMKENVASWPDFPANQDIIRPLSNPIKPSGHLQILRGSLAPGGSVGKITGKEGLRFEGTAKCYDYEDAFIESLERGEIKKGDKTVVIIRYEGPKGGPGMPEMLKPSAAIMGAGLGQDVALLTDGRFSGGSHGFLIGHIVPEAMEGGPIALARDGDRIVIDAEERVVDLDIPIEELEKRRKEWKAPPLRYQKGTLKKYCTLVSDASHGCVTDGPI

SEQ ID NO: 12 - protein, 644 aa, Penicillium brasilianum
MHPFLNKHGYLATNILLNSCLEHAGFCSSFHFFSYSTCVIPVHVSTGIMATSSIRSRALGLSRRARFETTRLPFIGRRYKSDETLNRISSKITQPKSQGASQAMLYATGLTEEDMSKAQVGISSVWFEGNPCNMHLNDLSGIVRDSVLRAGLVPMRFNSVGVSDGISMGTAGMRYSLQSRELIADGIETVMNAQWYDANISLPGCDKNMPGVLMAMGRTNRPSIMVYGGSIKPGCSAKGQKLDLVSAFQSYGQFITGQIDETERFDIIRNACPGKGACGGMYTANTLATAIETMGMTVPGSSSCPADDPKKLVECENIGEVVKNMLREEIKPRDVMTRQAFENAMIVVNVLGGSTNAVLHLIAIADSVGIKLTIDDFQAVSDKTPFLADLKPSGKYLMNDLYSIGGTPALLKYLLKEGLIDGSGITVTGKTMKENVASWPDFPADQDIIQPLSNPIKPSGHLQILRGSLAPGGSVGKITGKEGLRFEGTAKCYDYEDAFIESLERGEIKKGEKTVVIIRYEGPKGGPGMPEMLKPSAAIMGAGLGQDVALLTDGRFSGGSHGFLIGHIVPEAMEGGPIALARDGDRIVIDAEEKVVDLDVPTEELDARRKQWKAPPLRYQKGTLKKYCALVSDASHGCVTDGPI

SEQ ID NO: 13 - protein, 598 aa, Aspergillus brasiliensis
MFASNIRSRALGLSPRARFMNTRLPSSTSGRRYKSDETLNRISSKITQPKSQGASQAMLYATGLTEEDMSKPQVGISSVWFEGNPCNMHLHDLSAIVRDSVLRAGLVPMRFNSVGVSDGISMGTKGMRYSLQSRELIADGIETVMNAQWYDANVSLPGCDKNMPGVLMAMGRTNRPSIMVYGGSIKPGCSAKGQKLDLVSAFQSYGQFITGQIDEKERFDIIRNACPGRGACGGMYTANTLATAIETMGMTVPGSSSCPADDPKKLVECENIGEVVKAMLREDIKPRDILTRQAFENAMIVVNVLGGSTNAVLHLIAIADSVGIKLTIDDFQAVSDKTPFLADLKPSGKYLMNDLYNIGGTPALLKYLLKEGLIDGSGITVTGKTMKENVASWPDFPADQDIIRPLSNPIKPSGHLQILRGSLAPGGSVGKITGKEGLRFEGIAKCYDYEDAFIESLERGEIKKGEKTVVIIRYEGPKGGPGMPEMLKPSAAIMGAGLGQDVALLTDGRFSGGSHGFLIGHIVPEAMEGGPIALARDGDRIVIDAEERVVDLDIPTEELEKRRKEWKAPPLRYQKGTLKKYSTLVSDASHGCVTDGPI

SEQ ID NO: 14 - protein, 598 aa, Aspergillus niger
MFASSIRSRALGLSPRARFENTRLPSSTSGRRYRSDEPLNRISSKITQPKSQGASQAMLYATGLTEEDMSKPQVGISSVWFEGNPCNMHLHDLSAIVRDSVLRAGLVPMRFNSVGVSDGISMGTKGMRYSLQSRELIADGIETVMNAQWYDANVSLPGCDKNMPGVLIAMGRTNRPSIMVYGGSIKPGCSAKGQKLDLVSAFQSYGQFITGQIDEKERFDIIRNACPGRGACGGMYTANTLATAIETMGMTIPGSSSCPADDRKKLVECENIGEVVKNMLREDIKPRDILTRQAFENAMIVVNVLGGSTNAVLHLIAIADSVGIKLTIDDFQAVSDKTPFLADLKPSGKYLMNDLYNIGGTPALLKYLLKEGLIDGSGVTVTGKTMKENVASWPDFPADQDIIRPLNNPIKPSGHLQILRGSLAPGGSVGKITGKEGLRFEGIAKCYDYEDAFIESLERGEIKKGEKTVVIIRYEGPKGGPGMPEMLKPSAAIMGAGLGQDVALLTDGRFSGGSHGFLIGHIVPEAMEGGPIALARDGDRIVIDAEERVVDLDISTEELEKRRKEWNAPPLRYQKGTLKKYCTLVSDASHGCVTDGPI

SEQ ID NO: 15 - protein, 596 aa, Penicillium expansum
MATSSIRSRALGLSRRARFENTRLPLIGRRYKSDETLNRISSKITQPKSQGASQAMLYATGLTEEDMSKPQVGISSVWFEGNPCNMHLNDLSGIVRDSVLRAGLVPMRFNSVGVSDGISMGTAGMRYSLQSRELIADGIETVMNAQWYDANVSLPGCDKNMPGVLMAMGRTNRPSIMVYGGSIKPGCSAKGQKLDLVSAFQSYGQFITGQIDETERFDIIRNACPGKGACGGMYTANTLATAIETMGMTVPGSSSCPADDPKKLVECENIGEVVKQMLREEIKPRDIMTRQAFENAMIVVNVLGGSTNAVLHLIAIADSVGIKLTIDDFQAVSDKTPFLADLKPSGKYLMNDLYNIGGTPALLKYLLKEGLIDGSGITVTGKTMKENVASWPDFPADQEIIQPLSKPIKPSGHLQILRGSLAPGGSVGKITGKEGLRFEGTAKCYDYEDAFIESLERGEIKKGEKTVVIIRYEGPKGGPGMPEMLKPSAAIMGAGLGQDVALLTDGRFSGGSHGFLIGHIVPEAQEGGPIALARDGDRIVIDAEEKVVDLDVPTEELEKRRKEWKAPPLRYQKGTLKKYCALVSDASHGCVTDGPI

SEQ ID NO: 16 - protein, 633 aa, Aspergillus oryzae
MKGSPEFGPISGSLSCLQQVDFSFSLVSFPLHVSAAIMLSSNIRSRALGLSRRAQLQNTRLPPAGRRYKSDESLNRFSSKITQPKSQGASQAMLYATGLTEEDMSKPQVGISSVWFEGNPCNMHLNDLSGIVRDSVRRAGLVPMRFNSVGVSDGISMGTEGMRYSLQSRELIADGIESVMNGQWYDANVSLPGCDKNMPGVLMAMGRTNRPSIMVYGGSIKPGCSAKGQKLDLVSAFQSYGQYITGQIDEKERFDIIRNACPGRGACGGMYTANTLATAIETMGMTVPGSSSCPADDPKKLVECENIGEVVKNMLREDIRPSDVLTRQAFENAMIVVNILGGSTNAVLHLIAIADSVGIKLTIDDFQAVSDKTPFLADLKPSGKYVMNDLYTIGGTPALLRYLLKEGLIDGSGITVTGKTMKENVASWPDFPADQDIIHPLSKPIKPSGHLQILRGSLAPGGSVGKITGKEGLRFEGTAKCYDYEDAFIESLERGEIKKGEKTVVIIRYEGPKGGPGMPEMLKPSSAIMGAGLGQDVALLTDGRFSGGSHGFLIGHIVPEAIEGGPIALVRDGDRIVIDAEERVIDLDIPAEELEKRRKEWKAPPFRYQKGTLKKYATLVSDASHGCVTDGPI

SEQ ID NO: 17 - DNA, 1977 bp, Artificial Sequence
  Synthetic Construct
atgcaagccaccatcttctctccacgcgccactctcttcccctgtaaacctctcctcccttcccacaatgtcaactctcgccgtccctcaatcatctcctgctccgactacaaagacgatgacgacaaacacatggactacaaagacgatgacgacaaagactacaaagacgatgacgacaaattcgcatctcgtatccgatcaagagcccttggtcttcacccccgagctcgatttgaaaacactcgacttccggccagtactaccggaaggaggtataagagcgacgagaccctgaacagaattagctcaaaaatcactcagccgaagtcccagggggcatctcaggcgatgctctatgctaccggcttgacagaggaagacatgtcaaagccgcaggtcggaatctcatccgtttggtttgaggggaatccatgcaacatgcatcttcacgatttgtccgccatcgttcgtgactctgttcaccgagcaggtcttgtccccatgaggtttaattcagttggcgtttcagacgggatctctatgggtacgaaggggatgagatattccctccagtccagagaactgatagctgacggtattgagaccgtaatgaacgctcaatggtatgatgccaacgtgtctctgcctggctgtgacaaaaatatgccgggcgtcctcatggcgatgggtagaaccaatcgtccttccatcatggtctacggaggtagcatcaaacccggttgctctgccaagggacaaaaattagatctggtatctgcttttcaaagctatggacagttcataacgggtcagatagatgaaaaggaacgatttgatataattagaaacgcatgtcctggtcgtggagcttgcggtggaatgtacacggcaaacacactagctaccgctatagagactatgggtatgacagtgcccggctcttctagctgtccggcggatgaccctaaaaaactagtggagtgcgagaatataggcgaggtggtaaagacgatgctccgagaagatatcaaaccgcgagacgttctcacccgtcaggcttttgaaaatgcgatgattgtggtcaacatactagggggttctacaaatgccgtactccatctaatagccatagctgattccgtagggatcaaactgacgatagatgatttccaagccgtatctgataaaacaccgttcttggccgatctaaaaccctcagggaagtacttaatgaacgatttgtacaacatcggcggcaccccggcgcttttaaagtatctccttaaggaaggacttattgacggaagtggcataactgtcactggtaaaaccatgaaagaaaacgtggcctcttggcccgattttccctcagatcaagacataatccgaccgctctcaaacccgattaagccctccggccatttacaaattctcagggggtctctagcgccgggagggtcagtaggtaagattacgggtaaggaggggctcagatttgagggcaccgcaaagtgctatgactacgaggatgccttcatagagagtcttgagagaggtgagattaaaaagggagagaagacagtggtgataataaggtatgaaggcccaaaggggggcccgggcatgcctgaaatgctcaaaccaagcgccgcgattatgggtgcgggcttaggtcaagacgttgcacttctgacagatgggcgtttctcagggggatcacacggctttctaataggtcacattgtaccagaggcgatggaggggggtcccatagctttagcacgtgacggggatcgtattgtcatcgacgccgaggagcgagtagtcgatcttgagataccgaccgaagagttggagaaacgtcgaaaggagtggaaagcccccccacttcgataccaaaagggcacgctcaaaaaatattgcacgcttgttagcgatgcatctcacggttgcgtgacagacgggccgatttag

SEQ ID NO: 18 - DNA, 105 bp, Artificial Sequence
  Synthetic Construct
atgcaagccaccatcttctctccacgcgccactctcttcccctgtaaacctctcctcccttcccacaatgtcaactctcgccgtccctcaatcatctcctgctcc

SEQ ID NO: 19 - protein, 35 aa, Artificial Sequence
  Synthetic Construct
MQATIFSPRATLFPCKPLLPSHNVNSRRPSIISCS

SEQ ID NO: 20 - DNA, 78 bp, Artificial Sequence
  Synthetic Construct
gactacaaagacgatgacgacaaacacatggactacaaagacgatgacgacaaagactacaaagacgatgacgacaaa

SEQ ID NO: 21 - DNA, 1794 bp, Artificial Sequence
  Synthetic Construct
ttcgcatctcgtatccgatcaagagcccttggtcttcacccccgagctcgatttgaaaacactcgacttccggccagtactaccggaaggaggtataagagcgacgagaccctgaacagaattagctcaaaaatcactcagccgaagtcccagggggcatctcaggcgatgctctatgctaccggcttgacagaggaagacatgtcaaagccgcaggtcggaatctcatccgtttggtttgaggggaatccatgcaacatgcatcttcacgatttgtccgccatcgttcgtgactctgttcaccgagcaggtcttgtccccatgaggtttaattcagttggcgtttcagacgggatctctatgggtacgaaggggatgagatattccctccagtccagagaactgatagctgacggtattgagaccgtaatgaacgctcaatggtatgatgccaacgtgtctctgcctggctgtgacaaaaatatgccgggcgtcctcatggcgatgggtagaaccaatcgtccttccatcatggtctacggaggtagcatcaaacccggttgctctgccaagggacaaaaattagatctggtatctgcttttcaaagctatggacagttcataacgggtcagatagatgaaaaggaacgatttgatataattagaaacgcatgtcctggtcgtggagcttgcggtggaatgtacacggcaaacacactagctaccgctatagagactatgggtatgacagtgcccggctcttctagctgtccggcggatgaccctaaaaaactagtggagtgcgagaatataggcgaggtggtaaagacgatgctccgagaagatatcaaaccgcgagacgttctcacccgtcaggcttttgaaaatgcgatgattgtggtcaacatactagggggttctacaaatgccgtactccatctaatagccatagctgattccgtagggatcaaactgacgatagatgatttccaagccgtatctgataaaacaccgttcttggccgatctaaaaccctcagggaagtacttaatgaacgatttgtacaacatcggcggcaccccggcgcttttaaagtatctccttaaggaaggacttattgacggaagtggcataactgtcactggtaaaaccatgaaagaaaacgtggcctcttggcccgattttccctcagatcaagacataatccgaccgctctcaaacccgattaagccctccggccatttacaaattctcagggggtctctagcgccgggagggtcagtaggtaagattacgggtaaggaggggctcagatttgagggcaccgcaaagtgctatgactacgaggatgccttcatagagagtcttgagagaggtgagattaaaaagggagagaagacagtggtgataataaggtatgaaggcccaaaggggggcccgggcatgcctgaaatgctcaaaccaagcgccgcgattatgggtgcgggcttaggtcaagacgttgcacttctgacagatgggcgtttctcagggggatcacacggctttctaataggtcacattgtaccagaggcgatggaggggggtcccatagctttagcacgtgacggggatcgtattgtcatcgacgccgaggagcgagtagtcgatcttgagataccgaccgaagagttggagaaacgtcgaaaggagtggaaagcccccccacttcgataccaaaagggcacgctcaaaaaatattgcacgcttgttagcgatgcatctcacggttgcgtgacagacgggccgatttag

SEQ ID NO: 22 - protein, 604 aa, Chlamydomonas reinhardtii
MSSTATMPGQRSAMKAAGAQSRRAVKVMAVSAPEKPSSSAPAVPAGLNKFSSRITQPKYQGASQAMLFATGLREEDMIKPQVGISSVWYEGNPCNMHLMDLAAEVKKGVEAMGMVGFRFNTIGVSDGISMGTDGMSFSLQSRDLIADSIETVMSAQWYDANISLPGCDKNMPGTLMAMARLNRPSLMIYGGTIKPGHSRMDGSVLDIVSAFQSYGAYSAGLINEAQRVDIVRNSCPGAGACGGMYTANTMASAIEALGMTLPYSSSIPAEDPLKKDECRMAGRYMLELLKSDLKPLDIMTYKAFENAMVLVMATGGSTNAVLHFIAMARACGVPLTLDDFQRVSDRTPFICDLKPSGRYVMEDIHKVGGTPAVLKYLDSKGYINRDCMTVTGKTMGGNLAEVPELRAGQDVVLPVEKPIKQTGHIQILYGNLAPEGSVAKITGKEGLLFEGEALVFDNEEDMITMVGAEPNKFRGKVVVIRYEGPKGGPGMPEMLTPTSAIMGAGLGKECALITDGRFSGGSHGFVIGHVTPEAQVGGPIALVKNGDKIVIDVEKRVMDMKISDQELAARKAAWKAPPLKATSGTLYKYIKNVSSASTGCVTDS

SEQ ID NO: 23 - protein, 588 aa, Physcomitrella patens
MVVASSSAEGAVAAPPPQSVEAPAGSATDSAKLNKYSSRVTQPKAQGASQAILYGVGLSEEDMNKPQVGISSVWYEGNTCNMHLLHLSEAVKEGVKEAGMVGFRFNTVGVSDAVSMGTEGMCYSLQSRDLIADSVETVMGGQWYDANISIPGCDKNMPGVVMAMGRLNRPSIMIYGGTIKPGHFNGQTLDIVSAFQSYGEYVSGSISEDERMDVVRNSCPGFGACGGMYTANTMASAIEALGMSLPYSSSIPAEDPLKIEECKLAGKYILELLKRDLKPRDIITRKSLNNAMVVVMALGGSTNAVLHLIAIARSVGVELTLDDFQDVSDKTPFIADLKPSGKYVMEDLHKIGGVPAVLKYLLEKGLIDGSCMTVTGKTIAENLAECPPLSEGQKIIMPLENPIKKTGHLQILWGNLAPEGSVAKITGKEGLYFSGPARVFEGEEAMLDAITEDPQSLKGTVIVIRGEGPKGGPGMPEMLTPTSAVIGAGLGKEVALLTDGRFSGGSHGFVVGHICPEAQVGGPIGLVRDGDVITIDVEKRKINVDLTAQELADRKLLWRAPPYKASRGTLYKYIKNVKSASEGCVTDE

SEQ ID NO: 24 - protein, 605 aa, Populus euphratica
MQSTFVCRRATPLKPKTPFRTRLPPSSLLVKAQSVAVEPSQATSTAAQKLNKYSSRITEPKSQGGSQAILHGVGLSDDDMSKPQIGISSVWYEGNTCNMHLLKLSEAVKIGVEEAGMVGFRFNTIGVSDAISMGTRGMCYSLQSRDLIADSIETVMSAQWYDGNISIPGCDKNMPGTIMAMGRLNRPSIMVYGGTIKPGHFNGHTYDIISAFQVYGEYVSGSISDDERKNVVHNSCPGAGACGGMYTANTMASAIEALGMSLPYSSSIPAENQLKLDECRLAGKYLLELLKMDLKPRDIITRKSLRNAMVIVMALGGSTNAVLHLIAIARSVGLELTLDDFQKVSDEVPFLADLKPSGKYVMEDVHKIGGTPAVLRYLLEHGFLDGDCLTVTGKTLAENVQNCPPLSEGQEIIRSLENPIKQTGHLQILRGNLAPEGSVAKITGKEGLYFSGPALVFEGEESMIAAISEDPMSFKGKVVVIRGEGPKGGPGMPEMLTPTSAIMGAGLGKDCALLTDGRFSGGSHGFVAGHICPEAQEGGPIGLIRNGDVINVDIRERRIDVQLTDSELEERRKNWTPPPYKATRGVLYKYIKNVQSASEGCVTDE

SEQ ID NO: 25 - DNA, 60 bp, Artificial Sequence
  Synthetic Construct
gagagcctgagcttcatccccagcatcattacacctcagcaatgttcgcgtcgaggatcc

SEQ ID NO: 26 - DNA, 60 bp, Artificial Sequence
  Synthetic Construct
gactaaccattaccccgccacatagacacatctaaacaatggacatgaataccttccccg

SEQ ID NO: 27 - DNA, 60 bp, Artificial Sequence
  Synthetic Construct
gtggaggacatacccgtaattttctgggcatttaaatactccggtgaattgatttgggtg

SEQ ID NO: 28 - DNA, 25 bp, Artificial Sequence
  Synthetic Construct
tgtttagatgtgtctatgtggcggg

SEQ ID NO: 29 - DNA, 60 bp, Artificial Sequence
  Synthetic Construct
aaccattaccccgccacatagacacatctaaacaatgctattccaagacctgtcttttcc

SEQ ID NO: 30 - DNA, 60 bp, Artificial Sequence
  Synthetic Construct
gctaaagggtatcatcgaaagggagtcatccaggtactgcttgtattgaatcctagtttg

SEQ ID NO: 31 - DNA, 60 bp, Artificial Sequence
  Synthetic Construct
cccttctctgaacaataaaccccacagaaggcatttatgggagcttctactttctcccag

SEQ ID NO: 32 - DNA, 60 bp, Artificial Sequence
  Synthetic Construct
caacaaccatgataccaggggatttaaatttaattaaggttggggtttcatgcatatagc

SEQ ID NO: 33 - DNA, 60 bp, Artificial Sequence
  Synthetic Construct
tggctagcgattataaggatgatgatgataagactagtatggacatgaataccttccccg

SEQ ID NO: 34 - DNA, 60 bp, Artificial Sequence
  Synthetic Construct
atttgtcatttaaattagtgatggtgatggtgatgcacgtgttatgcgttgcctagcggg

SEQ ID NO: 35 - DNA, 60 bp, Artificial Sequence
  Synthetic Construct
caactatcaactattaactatatcgtaataccatatgctattccaagacctctcgtttcc

SEQ ID NO: 36 - DNA, 60 bp, Artificial Sequence
  Synthetic Construct
tacttgataatggaaactataaatcgtgaaggcatctacttgcagagacccataactcgc

SEQ ID NO: 37 - DNA, 60 bp, Artificial Sequence
  Synthetic Construct
atcaactatcaactattaactatatcgtaataccatatgggagcttctactttctccctg

SEQ ID NO: 38 - DNA, 60 bp, Artificial Sequence
  Synthetic Construct
ttgataatgaaaactataaatcgtgaaggcatgtttaaacctagcctcgtctctttattc

SEQ ID NO: 39 - DNA, 32 bp, Artificial Sequence
  Synthetic Construct
atagctagcatgcaagccaccatcttctctcc

SEQ ID NO: 40 - DNA, 37 bp, Artificial Sequence
  Synthetic Construct
atagcggccgcttactcgtcagtcacacatccatctg

SEQ ID NO: 41 - DNA, 27 bp, Artificial Sequence
  Synthetic Construct
atacatatgcttctctctcagacccgg

SEQ ID NO: 42 - DNA, 36 bp, Artificial Sequence
  Synthetic Construct
atagcggccgcttagtcaagagcatcggtgatgcag

SEQ ID NO: 43 - DNA, 25 bp, Artificial Sequence
  Synthetic Construct
atacatatgttcgcgtcgaggatcc

SEQ ID NO: 44 - DNA, 32 bp, Artificial Sequence
  Synthetic Construct
atagcggccgcctagatcggtccgtccgtgac

SEQ ID NO: 45 - DNA, 60 bp, Artificial Sequence
  Synthetic Construct
gcatagcaatctaatctaagttttaattacaaaactagtatgcttctctctcagacccgg

SEQ ID NO: 46 - DNA, 60 bp, Artificial Sequence
  Synthetic Construct
gaatgtaagcgtgacataactaattacatgactcgagttagtcaagagcatcggtgatgc

SEQ ID NO: 47 - DNA, 60 bp, Artificial Sequence
  Synthetic Construct
tagcaatctaatctaagttttaattacaaaactagtatggactacaaagacgatgacgac

SEQ ID NO: 48 - DNA, 60 bp, Artificial Sequence
  Synthetic Construct
gcgtgaatgtaagcgtgacataactaattacatgactcgagctagatcggtccgtccgtg

SEQ ID NO: 49 - DNA, 26 bp, Artificial Sequence
  Synthetic Construct
acaggatccgcccaatccgtaaccgc

SEQ ID NO: 50 - DNA, 32 bp, Artificial Sequence
  Synthetic Construct
cacgtcgacttactcgtcagtcacacatccat

SEQ ID NO: 51 - DNA, 39 bp, Artificial Sequence
  Synthetic Construct
acataggagcagcaagaatagacacacaagtctcacccg

SEQ ID NO: 52 - DNA, 41 bp, Artificial Sequence
  Synthetic Construct
gtctattcttgctgctcctatgtcaatggtgattatgtctc